European Patent Application EP 4 349 980 A2, published April 10, 2024. Title: Methods and Compositions for the Targeted Modification of a Genome. Applicant: Regeneron Pharmaceuticals, Inc. The sequence listing filed with the application follows.

SEQUENCE LISTING (94 sequences)

SEQ ID NO: 1 - skipped

SEQ ID NO: 2 - RNA, 80 nt, synthetic construct
  misc_feature 1..80: note = a guide RNA (gRNA)
  source 1..80: mol_type = other RNA
gttttagagctagaaatagcaagttaaaataaggctagtccgttatcaacttgaaaaagtggcaccgagtcggtgctttt

SEQ ID NO: 3 - RNA, 42 nt, synthetic construct
  misc_feature 1..42: note = a guide RNA (gRNA)
  source 1..42: mol_type = other RNA
gttttagagctagaaatagcaagttaaaataaggctagtccg

SEQ ID NO: 4 - RNA, 30 nt, synthetic construct
  misc_feature 1..30: note = a crRNA
  source 1..30: mol_type = other RNA
gttttagagctagaaatagcaagttaaaat

SEQ ID NO: 5 - RNA, 33 nt, synthetic construct
  misc_feature 1..33: note = a crRNA
  source 1..33: mol_type = other RNA
gttttagagctagaaatagcaagttaaaataag

SEQ ID NO: 6 - RNA, 26 nt, synthetic construct
  misc_feature 1..26: note = a crRNA
  source 1..26: mol_type = other RNA
gagtccgagcagaagaagaagtttta

SEQ ID NO: 7 - RNA, 12 nt, synthetic construct
  misc_feature 1..12: note = a tracrRNA
  source 1..12: mol_type = other RNA
aaggctagtccg

SEQ ID NO: 8 - RNA, 50 nt, synthetic construct
  misc_feature 1..50: note = a tracrRNA
  source 1..50: mol_type = other RNA
aaggctagtccgttatcaacttgaaaaagtggcaccgagtcggtgctttt

SEQ ID NO: 9 - protein, 203 aa, Mus musculus [sequence omitted]

SEQ ID NO: 10 - DNA, 15 bp, synthetic construct
  misc_feature 1..15: note = ZFN1a binding site
  source 1..15: mol_type = other DNA
caggccctgaaccgc

SEQ ID NO: 11 - skipped

SEQ ID NO: 12 - DNA, 16 bp, synthetic construct
  misc_feature 1..16: note = ZFN1b binding site
  source 1..16: mol_type = other DNA
gattacctgcgctggg

SEQ ID NO: 13 - DNA, 15 bp, synthetic construct
  misc_feature 1..15: note = ZF21a binding site
  source 1..15: mol_type = other DNA
ttcaccctccgcacc

SEQ ID NO: 14 - skipped

SEQ ID NO: 15 - DNA, 18 bp, synthetic construct
  misc_feature 1..18: note = ZF21b binding site
  source 1..18: mol_type = other DNA
tatccagatccaggggtt

SEQ ID NO: 16 - protein, 9 aa, synthetic construct
  REGION 1..9: note = conserved domain of a family of homing nucleases
LAGLIDADG

SEQ ID NO: 17 - DNA, 15 bp, synthetic construct
  misc_feature 1..15: note = ZFN1a binding site
  source 1..15: mol_type = other DNA
caggccctgaaccgc

SEQ ID NO: 18 - skipped

SEQ ID NO: 19 - DNA, 16 bp, synthetic construct
  misc_feature 1..16: note = ZFN1b binding site
  source 1..16: mol_type = other DNA
gattacctgcgctggg

SEQ ID NO: 20 - protein, 369 aa, Homo sapiens
MLKPSLPFTSLLFLQLPLLGVGLNTTILTPNGNEDTTADFFLTTMPTDSLSVSTLPLPEVQCFVFNVEYMNCTWNSSSEPQPTNLTLHYWYKNSDNDKVQKCSHYLFSEEITSGCQLQKKEIHLYQTFVVQLQDPREPRRQATQMLKLQNLVIPWAPENLTLHKLSESQLELNWNNRFLNHCLEHLVQYRTDWDHSWTEQSVDYRHKFSLPSVDGQKRYTFRVRSRFNPLCGSAQHWSEWSHPIHWGSNTSKENPFLFALEAVVISVGSMGLIISLLCVYFWLERTMPRIPTLKNLEDLVTEYHGNFSAWSGVSKGLAESLQPDYSERLCLVSEIPPKGGALGEGPGASPCNQHSPYWAPPCYTLKPET

SEQ ID NO: 21 - protein, 368 aa, Rattus norvegicus
MLKPLLPSRSFLLLQLLLLRVGWSSKVLMSSGNEDTKSDLLLTSMDLKHLSVPTLPLPEVQCFVFNVEYMNCTWNSSSEPQPTNLTMHYRYKGSDNNTFQECSHYLFSKEITSGCQIQKEDIQLYQTFVVQLQDPQKPQRRAEQKLNLQNLVIPWAPENLTLYNLSESQVELRWKSRYIERCLQYLVQYRSNRDRSWTEQIVDHEPRFSLPSVDEQKLYTFRVRSRFNPICGSTQQWSKWSQPIHWGSHTAEENPSLFALEAVLIPVGTMGLIITLIFVYCWLERMPRIPAIKNLEDLVTEYHGNFSAWSGVSKGLTESLQPDYSERFCHVSEIPPKGGALGEGPGGSPCSLHSPYWPPPCYSLKPEA

SEQ ID NO: 22 - protein, 368 aa, synthetic construct
  REGION 1..368: note = chimeric IL-2 receptor gamma comprising the rat IL-2 receptor gamma protein having the ecto domain of IL-2 gamma receptor from human
MLKPSLPFTSLLFLQLPLLGVGLNTTILTPNGNEDTTADFFLTTMPTDSLSVSTLPLPEVQCFVFNVEYMNCTWNSSSEPQPTNLTLHYWYKNSDNDKVQKCSHYLFSEEITSGCQLQKKEIHLYQTFVVQLQDPREPRRQATQMLKLQNLVIPWAPENLTLHKLSESQLELNWNNRFLNHCLEHLVQYRTDWDHSWTEQSVDYRHKFSLPSVDGQKRYTFRVRSRFNPLCGSAQHWSEWSHPIHWGSNTSKENPFLFALEAVLIPVGTMGLIITLIFVYCWLERMPRIPAIKNLEDLVTEYHGNFSAWSGVSKGLTESLQPDYSERFCHVSEIPPKGGALGEGPGGSPCSLHSPYWPPPCYSLKPEA

SEQ ID NO: 23 - skipped

SEQ ID NO: 24 - DNA, 20 bp, synthetic construct
  misc_feature 1..20: note = a guide sequence
  source 1..20: mol_type = other DNA
gggaacccacagcatactcc

SEQ ID NO: 25 - DNA, 20 bp, synthetic construct
  misc_feature 1..20: note = a guide sequence
  source 1..20: mol_type = other DNA
gaatcatgcacggctacccc

SEQ ID NO: 26 - DNA, 20 bp, synthetic construct
  misc_feature 1..20: note = a guide sequence
  source 1..20: mol_type = other DNA
tgctcctatggggaggcgcg

SEQ ID NO: 27 - DNA, 20 bp, synthetic construct
  misc_feature 1..20: note = a guide sequence
  source 1..20: mol_type = other DNA
cttggataacattgataccc

SEQ ID NO: 28 - DNA, 20 bp, synthetic construct
  misc_feature 1..20: note = a guide sequence
  source 1..20: mol_type = other DNA
ggggcagagcccttatatca

SEQ ID NO: 29 - DNA, 20 bp, synthetic construct
  misc_feature 1..20: note = a guide sequence
  source 1..20: mol_type = other DNA
tcgctcacattaatccctag

SEQ ID NO: 30 - DNA, 20 bp, synthetic construct
  misc_feature 1..20: note = a guide sequence
  source 1..20: mol_type = other DNA
gtactggggaatcggtggtc

SEQ ID NO: 31 - DNA, 20 bp, synthetic construct
  misc_feature 1..20: note = a guide sequence
  source 1..20: mol_type = other DNA
cacgcactccaaatttatcc

SEQ ID NO: 32 - DNA, 20 bp, synthetic construct
  misc_feature 1..20: note = a guide sequence
  source 1..20: mol_type = other DNA
ctaagtgtgtatcagtacat

SEQ ID NO: 33 - DNA, 20 bp, synthetic construct
  misc_feature 1..20: note = a guide sequence
  source 1..20: mol_type = other DNA
tgccctgcacaataagcgca

SEQ ID NO: 34 - DNA, 20 bp, synthetic construct
  misc_feature 1..20: note = a guide sequence
  source 1..20: mol_type = other DNA
actcattgaaacgttatggc

SEQ ID NO: 35 - DNA, 20 bp, synthetic construct
  misc_feature 1..20: note = a guide sequence
  source 1..20: mol_type = other DNA
agtaagggtggattaaattc

SEQ ID NO: 36 - DNA, 20 bp, synthetic construct
  misc_feature 1..20: note = a guide sequence
  source 1..20: mol_type = other DNA
gccatctagattcatgtaac

SEQ ID NO: 37 - DNA, 20 bp, synthetic construct
  misc_feature 1..20: note = a guide sequence
  source 1..20: mol_type = other DNA
gactagaaatgttctgcacc

SEQ ID NO: 38 - DNA, 20 bp, synthetic construct
  misc_feature 1..20: note = a guide sequence
  source 1..20: mol_type = other DNA
tgaaccaattgtgtagcctt

SEQ ID NO: 39 - DNA, 20 bp, synthetic construct
  misc_feature 1..20: note = a guide sequence
  source 1..20: mol_type = other DNA
aatagtggtaaagcaccatg

SEQ ID NO: 40 - DNA, 20 bp, synthetic construct
  misc_feature 1..20: note = a guide sequence
  source 1..20: mol_type = other DNA
gtgtgctaaggatcgaagtc

SEQ ID NO: 41 - DNA, 20 bp, synthetic construct
  misc_feature 1..20: note = a guide sequence
  source 1..20: mol_type = other DNA
caccgagatgcttgggtatt

SEQ ID NO: 42 - DNA, 20 bp, synthetic construct
  misc_feature 1..20: note = a guide sequence
  source 1..20: mol_type = other DNA
tgtaaccgccctgaatgacc

SEQ ID NO: 43 - DNA, 20 bp, synthetic construct
  misc_feature 1..20: note = a guide sequence
  source 1..20: mol_type = other DNA
aaaagggcatcataaatccc

SEQ ID NO: 44 - DNA, 20 bp, synthetic construct
  misc_feature 1..20: note = a guide sequence
  source 1..20: mol_type = other DNA
tcaaaaatagtcatacacct

SEQ ID NO: 45 - DNA, 20 bp, synthetic construct
  misc_feature 1..20: note = a guide sequence
  source 1..20: mol_type = other DNA
ggtctctagtacattgtaga

SEQ ID NO: 46 - DNA, 20 bp, synthetic construct
  misc_feature 1..20: note = a guide sequence
  source 1..20: mol_type = other DNA
atcacaaaccagttaaccgg

SEQ ID NO: 47 - DNA, 20 bp, synthetic construct
  misc_feature 1..20: note = a guide sequence
  source 1..20: mol_type = other DNA
tttcagacgagccgacccgg

SEQ ID NO: 48 - DNA, 20 bp, synthetic construct
  misc_feature 1..20: note = a guide sequence
  source 1..20: mol_type = other DNA
ctgtcaacagtgccgcgttt

SEQ ID NO: 49 - DNA, 20 bp, synthetic construct
  misc_feature 1..20: note = a guide sequence
  source 1..20: mol_type = other DNA
tgtgtgtcatagcgatgtcg

SEQ ID NO: 50 - DNA, 20 bp, synthetic construct
  misc_feature 1..20: note = a guide sequence
  source 1..20: mol_type = other DNA
aacaggtaccctatcctcac

SEQ ID NO: 51 - DNA, 20 bp, synthetic construct
  misc_feature 1..20: note = a guide sequence
  source 1..20: mol_type = other DNA
tcgtggttgcatgcgcactg

SEQ ID NO: 52 - DNA, 20 bp, synthetic construct
  misc_feature 1..20: note = a guide sequence
  source 1..20: mol_type = other DNA
ggcccggacctagtctctct

SEQ ID NO: 53 - DNA, 20 bp, synthetic construct
  misc_feature 1..20: note = a guide sequence
  source 1..20: mol_type = other DNA
agtctgtaaagttagcagtc

SEQ ID NO: 54 - DNA, 20 bp, synthetic construct
  misc_feature 1..20: note = a guide sequence
  source 1..20: mol_type = other DNA
ggtggtggtgctgacggaca

SEQ ID NO: 55 - DNA, 20 bp, synthetic construct
  misc_feature 1..20: note = a guide sequence
  source 1..20: mol_type = other DNA
tatgagatcaacactcgcta

SEQ ID NO: 56 - DNA, 20 bp, synthetic construct
  misc_feature 1..20: note = a guide sequence
  source 1..20: mol_type = other DNA
ccaaggacttccccacgtta

SEQ ID NO: 57 - DNA, 20 bp, synthetic construct
  misc_feature 1..20: note = a guide sequence
  source 1..20: mol_type = other DNA
tgcttcccttatgcaagatt

SEQ ID NO: 58 - DNA, 20 bp, synthetic construct
  misc_feature 1..20: note = a guide sequence
  source 1..20: mol_type = other DNA
ttaggtaccctatttgaata

SEQ ID NO: 59 - DNA, 20 bp, synthetic construct
  misc_feature 1..20: note = a guide sequence
  source 1..20: mol_type = other DNA
tgcagtgggtgacaggtcca

SEQ ID NO: 60 - DNA, 20 bp, synthetic construct
  misc_feature 1..20: note = a guide sequence
  source 1..20: mol_type = other DNA
agggttatactgacgttgtg

SEQ ID NO: 61 - DNA, 20 bp, synthetic construct
  misc_feature 1..20: note = a guide sequence
  source 1..20: mol_type = other DNA
tgtctttcaaggagggctac

SEQ ID NO: 62 - DNA, 20 bp, synthetic construct
  misc_feature 1..20: note = a guide sequence
  source 1..20: mol_type = other DNA
tgatgtgcagtcagacaaag

SEQ ID NO: 63 - DNA, 20 bp, synthetic construct
  misc_feature 1..20: note = a guide sequence
  source 1..20: mol_type = other DNA
tgcactatggttgactatga

SEQ ID NO: 64 - DNA, 20 bp, synthetic construct
  misc_feature 1..20: note = a guide sequence
  source 1..20: mol_type = other DNA
ggaatattctaataggaagt

SEQ ID NO: 65 - DNA, 20 bp, synthetic construct
  misc_feature 1..20: note = a guide sequence
  source 1..20: mol_type = other DNA
aagtgctgtaccattctagc

SEQ ID NO: 66 - DNA, 20 bp, synthetic construct
  misc_feature 1..20: note = a guide sequence
  source 1..20: mol_type = other DNA
taatcaatagacaacctcgt

SEQ ID NO: 67 - DNA, 20 bp, synthetic construct
  misc_feature 1..20: note = a guide sequence
  source 1..20: mol_type = other DNA
tcattcctaatggtattata

SEQ ID NO: 68 - DNA, 20 bp, synthetic construct
  misc_feature 1..20: note = a guide sequence
  source 1..20: mol_type = other DNA
agggtacatagatggcatcg

SEQ ID NO: 69 - DNA, 20 bp, synthetic construct
  misc_feature 1..20: note = a guide sequence
  source 1..20: mol_type = other DNA
ctctttaacaattaccactt

SEQ ID NO: 70 - DNA, 20 bp, synthetic construct
  misc_feature 1..20: note = a guide sequence
  source 1..20: mol_type = other DNA
tgtgggcctttgctgatcac

SEQ ID NO: 71 - DNA, 20 bp, synthetic construct
  misc_feature 1..20: note = a guide sequence
  source 1..20: mol_type = other DNA
aatctatgatcctatggcct

SEQ ID NO: 72 - DNA, 20 bp, synthetic construct
  misc_feature 1..20: note = a guide sequence
  source 1..20: mol_type = other DNA
tgccaatagcagtgacttga

SEQ ID NO: 73 - DNA, 20 bp, synthetic construct
  misc_feature 1..20: note = a guide sequence
  source 1..20: mol_type = other DNA
gggaagaatgggctattgtc

SEQ ID NO: 74 - DNA, 20 bp, synthetic construct
  misc_feature 1..20: note = a guide sequence
  source 1..20: mol_type = other DNA
ggttgtttgtgctgatgacg

SEQ ID NO: 75 - DNA, 20 bp, synthetic construct
  misc_feature 1..20: note = a guide sequence
  source 1..20: mol_type = other DNA
ccgtcctaggccttctacgt

SEQ ID NO: 76 - DNA, 20 bp, synthetic construct
  misc_feature 1..20: note = a guide sequence
  source 1..20: mol_type = other DNA
actagtagacctgaggggtt

SEQ ID NO: 77 - DNA, 20 bp, synthetic construct
  misc_feature 1..20: note = a guide sequence
  source 1..20: mol_type = other DNA
gctccagtgtttaggccttg

SEQ ID NO: 78 - DNA, 20 bp, synthetic construct
  misc_feature 1..20: note = a guide sequence
  source 1..20: mol_type = other DNA
ggcaagctgaaaacgcatgc

SEQ ID NO: 79 - DNA, 20 bp, synthetic construct
  misc_feature 1..20: note = a guide sequence
  source 1..20: mol_type = other DNA
gtagatcgctttccactacc

SEQ ID NO: 80 - DNA, 20 bp, synthetic construct
  misc_feature 1..20: note = a guide sequence
  source 1..20: mol_type = other DNA
gaactccactgctcgtgagc

SEQ ID NO: 81 - DNA, 20 bp, synthetic construct
  misc_feature 1..20: note = a guide sequence
  source 1..20: mol_type = other DNA
ataggtgggcactattgaag

SEQ ID NO: 82 - DNA, 20 bp, synthetic construct
  misc_feature 1..20: note = a guide sequence
  source 1..20: mol_type = other DNA
atgggaaggtttataccagc

SEQ ID NO: 83 - DNA, 20 bp, synthetic construct
  misc_feature 1..20: note = a guide sequence
  source 1..20: mol_type = other DNA
cggtgtaaaaacaacgggaa

SEQ ID NO: 84 - RNA, 20 nt, synthetic construct
  misc_feature 1..20: note = a guide sequence
  source 1..20: mol_type = other RNA
gacccgcagtcccagcgtcg

SEQ ID NO: 85 - DNA, 20 bp, synthetic construct
  misc_feature 1..20: note = a guide sequence
  source 1..20: mol_type = other DNA
actgagatcaatgaccccga

SEQ ID NO: 86 - DNA, 20 bp, synthetic construct
  misc_feature 1..20: note = a guide sequence
  source 1..20: mol_type = other DNA
gggtcgcccggaacctctac

SEQ ID NO: 87 - DNA, 23 bp, synthetic construct
  misc_feature 1..23: note = a guide sequence
  source 1..23: mol_type = other DNA
gcaggccctgaaccgcttcttgg

SEQ ID NO: 88 - DNA, 23 bp, synthetic construct
  misc_feature 1..23: note = a guide sequence
  source 1..23: mol_type = other DNA
cctgcgctgggtgcagacgcttt

SEQ ID NO: 89 - DNA, 20 bp, synthetic construct
  misc_feature 1..20: note = a guide sequence
  source 1..20: mol_type = other DNA
ccagctacttgctcgtacaa

SEQ ID NO: 90 - DNA, 20 bp, synthetic construct
  misc_feature 1..20: note = a guide sequence
  source 1..20: mol_type = other DNA
cccctcagattcacgtgcgt

SEQ ID NO: 91 - DNA, 23 bp, synthetic construct
  misc_feature 1..23: note = a guide sequence
  source 1..23: mol_type = other DNA
gaagctctttctatacaatctgg

SEQ ID NO: 92 - DNA, 23 bp, synthetic construct
  misc_feature 1..23: note = a guide sequence
  source 1..23: mol_type = other DNA
cccccgaaaggaggagccctagg

SEQ ID NO: 93 - DNA, 56 bp, Rattus norvegicus
  source 1..56: mol_type = genomic DNA
ttctgagcctcagccgaccaacctcactatgcactataggtatgagaagggggagg

SEQ ID NO: 94 - DNA, 20 bp, synthetic construct
  misc_feature 1..20: note = a guide sequence
  source 1..20: mol_type = other DNA
gtatagccctgttacacatt